European Patent Specification EP 3 481 948 B1, published November 1, 2023. Title: XYLANASE VARIANTS AND POLYNUCLEOTIDES ENCODING SAME. Applicant: Novozymes A/S Danielsen, Steffen Hansen, Peter Kamp Rasmussen, Frank Winther Pache, Roland Alexander. The sequence listing filed with the application follows.

SEQUENCE LISTING (6 sequences)

SEQ ID NO: 1 - protein, 391 aa, Bacillus subtilis
AASDVTVNVSAEKQVIRGFGGMNHPAWAGDLTAAQRETAFGNGQNQLGFSILRIHVDENRNNWYKEVETAKSAVKHGAIVFASPWNPPSDMVETFNRNGDTSAKRLKYNKYAAYAQHLNDFVTFMKNNGVNLYAISVQNEPDYAHEWTWWTPQEILRFMRENAGSINARVIAPESFQYLKNLSDPILNDPQALANMDILGTHLYGTQVSQFPYPLFKQKGAGKDLWMTEVYYPNSDTNSADRWPEALDVSQHIHNAMVEGDFQAYVWWYIRRSYGPMKEDGTISKRGYNMAHFSKFVRPGYVRIDATKNPNANVYVSAYKGDNKVVIVAINKSNTGVNQNFVLQNGSASNVSRWITSSSSNLQPGTNLTVSGNHFWAHLPAQSVTTFVVNR

SEQ ID NO: 2 - protein, 391 aa, Bacillus amyloliquefaciens
AANDVTVNISAERQVIRGFGGMNHPAWVGDLTAAQRETAFGNGQNQLGFSILRIHVDENRNNWYKEVETAKSAIKHGAIVFASPWNPPNDMVETFNHNGDTSAKRLRYDKYAAYAQHLNDFVNFMKSNGVNLYAISIQNEPDYAHEWTWWTPQEILRFMRENAGSINARVIAPESFQYLKNLSDPILNDPQALANMDILGTHLYGTQVSQFPYPLFKQKGAGKDLWMTEVYYPNSDNNSADRWPEALDVSQHIHSSMVEGDLQAYVWWYIRRSYGPMKEDGTISKRGYNMAHFSKFVRPGYVRIDATKNPNPNVYVSAYKGDNKVVIVAINKTNTGVNQNFVLQNGSASQVSRWITSSNSNLQPGTDLKVTDNHFWAHLPAQSVTTFVVKR

SEQ ID NO: 3 - protein, 392 aa, Bacillus licheniformis
AASDATVRLSAEKQVIRGFGGMNHPAWIGDLTAAQRETAFGNGQNQLGFSILRIHVDENRNNWYREVETAKSAIKHGAIVFASPWNPPSDMVETFNRNGDTSAKRLRYDKYAAYAKHLNDFVTFMKNNGVNLYAISVQNEPDYAHDWTWWTPQEILRFMKENAGSINARVIAPESFQYLKNISDPIVNDPKALANMDILGAHLYGTQLNNFAYPLFKQKGAGKDLWMTEVYYPNSDNHSADRWPEALDVSHHIHNSMVEGDFQAYVWWYIRRSYGPMKEDGTISKRGYNMAHFSKFVRPGYVRVDATKSPASNVYVSAYKGDNKVVIVAINKNNSGVNQNFVLQNGSVSQVSRWITSSSSNLQPGTNLNVTDNHFWAHLPAQSVTTFVANLR

SEQ ID NO: 4 - protein, 391 aa, Bacillus subtilis
AANDVTVNISAEKQVIRGFGGMNHPAWVGDLTAAQRETAFGNGQNQLGFSILRIHVDENRNNWYKEVETAKSAIKHGAIVFASPWNPPSNMVETFNHNGDTSAKRLRYDKYAAYAQHLNDFVTFMKSNGVNLYAISIQNEPDYAHEWTWWTPQEILRFMRENAGSINARVIAPESFQYLKNLSDPILNDPQALANMDILGTHLYGTQVSQFPYPLFKQKGAGKDLWMTEVYYPNSDNNSADRWPEALDVSQHIHNSMVEGDFQAYVWWYIRRSYGPMKEDGTISKRGYNMAHFSKFVRPGYVRIDATKNPNPNVYVSAYKGDNKVVIVAINKSNTGVNQNFVLQNGSASQVSRWITSSNSNLQPGTNLKVTDNHFWAHLPAQSVTTFVVIR

SEQ ID NO: 5 - protein, 393 aa, Paenibacillus pabuli
AASDVTVNLSSEKQLIKGFGGINHPNWIGDLTPSQRDTAFGNGQNQLGFSILRIYIDDNKNNWYKEIPTAKRAIEQGAIVFASPWNPPSDMVETFNRNGDTAAKRLKYDKYAAYAQHLNDFVSYMKSNGVNLYAISVQNEPDYAHDWTWWTPQEMLRFMKDYAGSITGTKVMAPESFSYLKEMSDPILNDPQALANMDILGAHTYGTQFSNFPYPLFKQKGAGKELWMSEVYYPNSNANSADHWPEALDVSYHIHHAMVEADFQAYVWWYIRRQYGPMKEDGTISKRGYNMAHFSKFVRPGFVRVDATKNPDTQTFISAFKGDNKVVIVAINRGTSAVNQKFVLQNGNASNVSSWVTDSTRNLAAGSSIIMTGNTFTAQLPSQSVTTFVAQLN

SEQ ID NO: 6 - protein, 391 aa, Bacillus amyloliquefaciens
AASDATVNISAERQVIRGFGGMNHPAWIGDLTAPQRVTAFGNGQNQLGFSVLRIHVDENRNNWYKEVETAKSAIKHGAIVFASPWNPPNDMVETFNHNGDTSAKRLRYDKYAAYAQHLNDFVNFMKSNGVNLYAISMQNEPDYAHEWTWWTPQEILRFMRENAGSINTRVIAPESFQYLKNISDPILNDPQALRNMDILGTHLYGTQVSQFPYPLFKQKGGGKELWMTEVYYPNSDNYSADRWPEALGVSEHIHHSMVEGDFQAYVWWYIRRSYGPMKEDGMISKRGYNMAHFSKFVRPGYVRIDATKNPEPNVYVSAYKGDNKVVIVAINKNNTGVNQNFVLQNGTASQVSRWITSSSSNLQPGTDLKVTDNHFWAHLPAQSVTTFVVKR